European Patent Application EP 4 260 870 A1, published October 18, 2023. Title: PRAME binding molecule. Applicant: MIE UNIVERSITY. The sequence listing filed with the application follows.

SEQUENCE LISTING (30 sequences)

SEQ ID NO: 1 - protein, 8 aa, Artificial Sequence
  H CDR1
GGTFSSYA

SEQ ID NO: 2 - protein, 8 aa, Artificial Sequence
  H CDR2
IIPIFGTA

SEQ ID NO: 3 - protein, 14 aa, Artificial Sequence
  H CDR3
ARHHSNYYYYGMDV

SEQ ID NO: 4 - protein, 121 aa, Artificial Sequence
  H variable region
QVQLVQSGAEVKKPGSSVKVSCKASGGTFSSYAISWVRQAPGQGLEWMGGIIPIFGTANYAQKFQGRVTITADESTGTAYMELSSLRSEDTAVYYCARHHSNYYYYGMDVWGQGTTVTVSR

SEQ ID NO: 5 - DNA, 24 bp, Artificial Sequence
  H CDR1
ggaggcaccttcagcagctatgct

SEQ ID NO: 6 - DNA, 24 bp, Artificial Sequence
  H CDR2
atcatccctatctttggtacagca

SEQ ID NO: 7 - DNA, 42 bp, Artificial Sequence
  H CDR3
gcgagacaccacagtaactactactactacggtatggacgtc

SEQ ID NO: 8 - DNA, 363 bp, Artificial Sequence
  H variable region
caggtgcagctggtgcagtctggggctgaggtgaagaagcctgggtcctcggtgaaggtctcctgcaaggcttctggaggcaccttcagcagctatgctatcagctgggtgcgacaggcccctggacaagggcttgagtggatgggagggatcatccctatctttggtacagcaaactacgcacagaagttccagggcagagtcacgattaccgcggacgaatccacgggcacagcctacatggagctgagcagcctgagatctgaggacacggccgtgtattactgtgcgagacaccacagtaactactactactacggtatggacgtctggggccaagggaccacggtcaccgtctcgaga

SEQ ID NO: 9 - protein, 6 aa, Artificial Sequence
  L CDR1
NIGSKN

SEQ ID NO: 10 - protein, 3 aa, Artificial Sequence
  L CDR2
RDS

SEQ ID NO: 11 - protein, 8 aa, Artificial Sequence
  L CDR3
QVWDSSHV

SEQ ID NO: 12 - protein, 105 aa, Artificial Sequence
  L variable region
SYELTQPLSVSVALGQTARITCGGNNIGSKNVHWYQQKPGQAPVLVIYRDSNRPSGIPERFSGSNSGNTATLTISRAQAGDEADYYCQVWDSSHVFGTGTKVTVL

SEQ ID NO: 13 - DNA, 18 bp, Artificial Sequence
  L CDR1
aacattggaagtaaaaat

SEQ ID NO: 14 - DNA, 9 bp, Artificial Sequence
  L CDR2
agggatagc

SEQ ID NO: 15 - DNA, 24 bp, Artificial Sequence
  L CDR3
caggtgtgggacagcagccatgtc

SEQ ID NO: 16 - DNA, 315 bp, Artificial Sequence
  L variable region
tcctatgagctgactcagccactctcagtgtcagtggccctgggacagacggccaggattacctgtggcggaaacaacattggaagtaaaaatgtgcactggtaccagcagaagccaggccaggcccctgtgctggtcatctatagggatagcaaccggccctctgggatccctgagcgattctctggctccaactcggggaacacggccaccctgaccatcagcagagcccaagccggggatgaggctgactattactgtcaggtgtgggacagcagccatgtcttcggaactgggaccaaggtcaccgtccta

SEQ ID NO: 17 - protein, 9 aa, Artificial Sequence
  PRAMEp301-309
LYVDSLFFL

SEQ ID NO: 18 - protein, 9 aa, Artificial Sequence
  PRAME p301-1A
AYVDSLFFL

SEQ ID NO: 19 - protein, 9 aa, Artificial Sequence
  PRAME p301-2A
LAVDSLFFL

SEQ ID NO: 20 - protein, 9 aa, Artificial Sequence
  PRAME p301-3A
LYADSLFFL

SEQ ID NO: 21 - protein, 9 aa, Artificial Sequence
  PRAME p301-4A
LYVASLFFL

SEQ ID NO: 22 - protein, 9 aa, Artificial Sequence
  PRAME p301-5A
LYVDALFFL

SEQ ID NO: 23 - protein, 9 aa, Artificial Sequence
  PRAME p301-6A
LYVDSAFFL

SEQ ID NO: 24 - protein, 9 aa, Artificial Sequence
  PRAME p301-7A
LYVDSLAFL

SEQ ID NO: 25 - protein, 9 aa, Artificial Sequence
  PRAME p301-8A
LYVDSLFAL

SEQ ID NO: 26 - protein, 9 aa, Artificial Sequence
  PRAME p301-9A
LYVDSLFFA

SEQ ID NO: 27 - protein, 9 aa, Artificial Sequence
  PRAME p301-2W
LWVDSLFFL

SEQ ID NO: 28 - protein, 9 aa, Artificial Sequence
  PRAME p301-2F
LFVDSLFFL

SEQ ID NO: 29 - protein, 9 aa, Artificial Sequence
  PRAME p301-9F
LYVDSLFFF

SEQ ID NO: 30 - protein, 9 aa, Artificial Sequence
  PRAME p301-9I
LYVDSLFFI